European Patent Application EP 4 814 016 A1, published September 30, 2026. Title: Antibody or fragment thereof specifically binding to glycoprotein 100. Applicant: Eberhard Karls Universität Tübingen - Medizinische Fakultät. Application EP. The sequence listing filed with the application follows.

SEQUENCE LISTING (48 sequences)

SEQ ID NO: 1 - protein, 5 aa, synthetic construct
SYEMH

SEQ ID NO: 2 - protein, 17 aa, synthetic construct
GMSYDGSKTFHSESVKG

SEQ ID NO: 3 - protein, 15 aa, synthetic construct
FNYYDGSGSMPGFDL

SEQ ID NO: 4 - protein, 12 aa, synthetic construct
RASQSVGSNYLA

SEQ ID NO: 5 - protein, 7 aa, synthetic construct
GASSRAA

SEQ ID NO: 6 - protein, 10 aa, synthetic construct
HQYGRSRDYI

SEQ ID NO: 7 - protein, 29 aa, synthetic construct
VQLVEAGGGAVQTGKSLRLSCVASGFGFS

SEQ ID NO: 8 - protein, 14 aa, synthetic construct
WVRQAPGKGLEWVA

SEQ ID NO: 9 - protein, 32 aa, synthetic construct
RLTISRDNSKNTLYLQMNSLRGEDTALYFCAR

SEQ ID NO: 10 - protein, 11 aa, synthetic construct
WGQGTMVIVSS

SEQ ID NO: 11 - protein, 123 aa, synthetic construct
VQLVEAGGGAVQTGKSLRLSCVASGFGFSSYEMHWVRQAPGKGLEWVAGMSYDGSKTFHSESVKGRLTISRDNSKNTLYLQMNSLRGEDTALYFCARFNYYDGSGSMPGFDLWGQGTMVIVSS

SEQ ID NO: 12 - protein, 16 aa, synthetic construct
PVTLSLSPGERATLSC

SEQ ID NO: 13 - protein, 15 aa, synthetic construct
WFQQKPGQAPRLLIY

SEQ ID NO: 14 - protein, 32 aa, synthetic construct
GIPDRFSGSGSGTDFTLTISSLEPEDFAVYYC

SEQ ID NO: 15 - protein, 10 aa, synthetic construct
FGQGTKVDIK

SEQ ID NO: 16 - protein, 102 aa, synthetic construct
PVTLSLSPGERATLSCRASQSVGSNYLAWFQQKPGQAPRLLIYGASSRAAGIPDRFSGSGSGTDFTLTISSLEPEDFAVYYCHQYGRSRDYIFGQGTKVDIK

SEQ ID NO: 17 - protein, 5 aa, synthetic construct
TYSMN

SEQ ID NO: 18 - protein, 17 aa, synthetic construct
SISDTSIYMYYVDSVQG

SEQ ID NO: 19 - protein, 14 aa, synthetic construct
SRPSRISAQFGMDV

SEQ ID NO: 20 - protein, 11 aa, synthetic construct
RASQSISNYLN

SEQ ID NO: 21 - protein, 7 aa, synthetic construct
AASSLHS

SEQ ID NO: 22 - protein, 9 aa, synthetic construct
QQSNSFPLT

SEQ ID NO: 23 - protein, 29 aa, synthetic construct
VQLVESGGGLVKPGGSLRLSCVASGFTFS

SEQ ID NO: 24 - protein, 14 aa, synthetic construct
WVRQAPGKGLEWVS

SEQ ID NO: 25 - protein, 32 aa, synthetic construct
RFTISRDNAKNSLYLQMNSLRVDDTAVYYCAR

SEQ ID NO: 26 - protein, 11 aa, synthetic construct
WGQGTTVTVSS

SEQ ID NO: 27 - protein, 122 aa, synthetic construct
VQLVESGGGLVKPGGSLRLSCVASGFTFSTYSMNWVRQAPGKGLEWVSSISDTSIYMYYVDSVQGRFTISRDNAKNSLYLQMNSLRVDDTAVYYCARSRPSRISAQFGMDVWGQGTTVTVSS

SEQ ID NO: 28 - protein, 16 aa, synthetic construct
PFSLSASVGDRVTITC

SEQ ID NO: 29 - protein, 15 aa, synthetic construct
WYQREPGKAPKILIY

SEQ ID NO: 30 - protein, 32 aa, synthetic construct
GVPSRFSGSGSGTEFTLTISGLQPEDSAIYFC

SEQ ID NO: 31 - protein, 9 aa, synthetic construct
FGGGTKVEI

SEQ ID NO: 32 - protein, 99 aa, synthetic construct
PFSLSASVGDRVTITCRASQSISNYLNWYQREPGKAPKILIYAASSLHSGVPSRFSGSGSGTEFTLTISGLQPEDSAIYFCQQSNSFPLTFGGGTKVEI

SEQ ID NO: 33 - protein, 5 aa, synthetic construct
DYDMN

SEQ ID NO: 34 - protein, 19 aa, synthetic construct
FIRGKAYGGTTEYAASVKG

SEQ ID NO: 35 - protein, 21 aa, synthetic construct
GFRRVVKHYFDSSGYFGKFDF

SEQ ID NO: 36 - protein, 11 aa, synthetic construct
RASQGIRNDLG

SEQ ID NO: 37 - protein, 7 aa, synthetic construct
AASSLQS

SEQ ID NO: 38 - protein, 9 aa, synthetic construct
LQHNNYPWT

SEQ ID NO: 39 - protein, 30 aa, synthetic construct
EVQLVESGGGLVKPGRSLRLSCTTSGFTFG

SEQ ID NO: 40 - protein, 14 aa, synthetic construct
WFRQAPGKGLEWVG

SEQ ID NO: 41 - protein, 32 aa, synthetic construct
RFTISRDDSKSVAYLQMNSLKTEDTAVYYCTR

SEQ ID NO: 42 - protein, 11 aa, synthetic construct
WGQGTLVTVSS

SEQ ID NO: 43 - protein, 132 aa, synthetic construct
EVQLVESGGGLVKPGRSLRLSCTTSGFTFGDYDMNWFRQAPGKGLEWVGFIRGKAYGGTTEYAASVKGRFTISRDDSKSVAYLQMNSLKTEDTAVYYCTRGFRRVVKHYFDSSGYFGKFDFWGQGTLVTVSS

SEQ ID NO: 44 - skipped

SEQ ID NO: 45 - protein, 15 aa, synthetic construct
WYQQKPGKAPKRLIY

SEQ ID NO: 46 - protein, 32 aa, synthetic construct
GVPSRFSGSGSGTEFTLTISSLQPEDFATYYC

SEQ ID NO: 47 - protein, 10 aa, synthetic construct
FGQGTKVEIK

SEQ ID NO: 48 - protein, 100 aa, synthetic construct
PVSLSASVGDRVTITCRASQGIRNDLGWYQQKPGKAPKRLIYAASSLQSGVPSRFSGSGSGTEFTLTISSLQPEDFATYYCLQHNNYPWTFGQGTKVEIK